European Patent Application EP 4 446 335 A1, published October 16, 2024. Title: A novel peptide and use thereof. Applicant: RUDACURE CORPORATION. The sequence listing filed with the application follows.

SEQUENCE LISTING (53 sequences)

SEQ ID NO: 1 - protein, 12 aa, synthetic construct
MLYFNDKQQIIY

SEQ ID NO: 2 - protein, 19 aa, synthetic construct
PINMLYFNDKQQIIYGKID

SEQ ID NO: 3 - protein, 19 aa, synthetic construct
GINMLYFNDKQQIIYGKIN

SEQ ID NO: 4 - protein, 13 aa, synthetic construct
YCSGQCYMFMQKY

SEQ ID NO: 5 - protein, 11 aa, synthetic construct
YKANYCSGQCY

SEQ ID NO: 6 - protein, 11 aa, synthetic construct
SGQCYMFMQKY

SEQ ID NO: 7 - protein, 12 aa, synthetic construct
YKANYCSGQCEY

SEQ ID NO: 8 - protein, 12 aa, synthetic construct
SGQCEYMFMQKY

SEQ ID NO: 9 - protein, 11 aa, synthetic construct
AGQCYMFMQKY

SEQ ID NO: 10 - protein, 11 aa, synthetic construct
SGQAYMFMQKY

SEQ ID NO: 11 - protein, 11 aa, synthetic construct
YGQCYMWMQKW

SEQ ID NO: 12 - protein, 11 aa, synthetic construct
YGQCYMYMQKW

SEQ ID NO: 13 - protein, 11 aa, synthetic construct
YGQCYMWMQYW

SEQ ID NO: 14 - protein, 11 aa, synthetic construct
YGQCYMWMQWW

SEQ ID NO: 15 - protein, 11 aa, synthetic construct
YGQCYMWMQGW

SEQ ID NO: 16 - protein, 11 aa, synthetic construct
YGQCYMWMQKY

SEQ ID NO: 17 - protein, 11 aa, synthetic construct
YGQCYMWMQEW

SEQ ID NO: 18 - protein, 11 aa, synthetic construct
YGMCYMWMQKW

SEQ ID NO: 19 - protein, 11 aa, synthetic construct
YGRCYMWMQKW

SEQ ID NO: 20 - protein, 11 aa, synthetic construct
YGQCYMWFQKW

SEQ ID NO: 21 - protein, 11 aa, synthetic construct
YGICYMWMQKW

SEQ ID NO: 22 - protein, 11 aa, synthetic construct
YGQCYMWMQHW

SEQ ID NO: 23 - protein, 11 aa, synthetic construct
YGQCYMWYQKW

SEQ ID NO: 24 - protein, 11 aa, synthetic construct
YGQCYMWSQKW

SEQ ID NO: 25 - protein, 11 aa, synthetic construct
YGGCYMWMQKW

SEQ ID NO: 26 - protein, 11 aa, synthetic construct
YKQCYMWMQKW

SEQ ID NO: 27 - protein, 11 aa, synthetic construct
YGTCYMWMQKW

SEQ ID NO: 28 - protein, 11 aa, synthetic construct
YGQCYMWGQKW

SEQ ID NO: 29 - protein, 11 aa, synthetic construct
YGQCYMWMQSW

SEQ ID NO: 30 - protein, 11 aa, synthetic construct
YGQCYMWMQCW

SEQ ID NO: 31 - protein, 11 aa, synthetic construct
YGQCYMWMQAW

SEQ ID NO: 32 - protein, 11 aa, synthetic construct
YGQWYMWMQKW

SEQ ID NO: 33 - protein, 11 aa, synthetic construct
YGQMYMWMQKW

SEQ ID NO: 34 - protein, 11 aa, synthetic construct
YGLCYMWMQKW

SEQ ID NO: 35 - protein, 11 aa, synthetic construct
YGQCYMWHQKW

SEQ ID NO: 36 - protein, 11 aa, synthetic construct
YSQCYMWMQKW

SEQ ID NO: 37 - protein, 11 aa, synthetic construct
YGQCYMWMQMW

SEQ ID NO: 38 - protein, 11 aa, synthetic construct
YGQPYMWMQKW

SEQ ID NO: 39 - protein, 11 aa, synthetic construct
YGQCYMWPQKW

SEQ ID NO: 40 - protein, 11 aa, synthetic construct
YGQGYMWMQKW

SEQ ID NO: 41 - protein, 11 aa, synthetic construct
YGSCYMWMQKW

SEQ ID NO: 42 - protein, 11 aa, synthetic construct
YLQCYMWMQKW

SEQ ID NO: 43 - protein, 11 aa, synthetic construct
YKAAYCSGQCY

SEQ ID NO: 44 - protein, 11 aa, synthetic construct
SGACYMFMQKY

SEQ ID NO: 45 - protein, 11 aa, synthetic construct
SGQCYAFMQKY

SEQ ID NO: 46 - protein, 11 aa, synthetic construct
SGQCYMFMQAY

SEQ ID NO: 47 - protein, 11 aa, synthetic construct
SGQCYMWMQKY

SEQ ID NO: 48 - protein, 11 aa, synthetic construct
SGQCYMWMQKW

SEQ ID NO: 49 - protein, 11 aa, synthetic construct
SGQCYMYMQKY

SEQ ID NO: 50 - protein, 109 aa, synthetic construct
NLGLDCDEHSSESRCCRYPLTVDFEAFGWDWIIAPKRYKANYCSGQCEYMFMQKYPHTHLVQQANPRGSAGPCCTPTKMSPINMLYFNDKQQIIYGKIPGMVVDRCGCS

SEQ ID NO: 51 - protein, 11 aa, synthetic construct
LYFNDKQQIIY

SEQ ID NO: 52 - protein, 15 aa, synthetic construct
NMLYFNDKQQIIYGK

SEQ ID NO: 53 - protein, 19 aa, synthetic construct
PINMLYFNDKQQIIYGKIP